European Patent Application EP 4 186 919 A1, published May 31, 2023. Title: SELF-COMPLEMENTARY ADENO-ASSOCIATED VIRUS VECTOR AND ITS USE IN TREATMENT OF MUSCULAR DYSTROPHY. Applicant: Research Institute at Nationwide Children's Hospital. The sequence listing filed with the application follows.

SEQUENCE LISTING (11 sequences)

SEQ ID NO: 1 - DNA, 4857 bp, synthetic construct
  misc_feature 1..4857: note = scAAV construct sequence
  source 1..4857: mol_type = other DNA
ctgcgcgctcgctcgctcactgaggccgcccgggcaaagcccgggcgtcgggcgacctttggtcgcccggcctcagtgagcgagcgagcgcgcagagagggagtggccaactccatcactaggggttccttgtagttaatgattaacccgccatgctacttatctacgtagccatgctctagaggcgcgcccctgcaggacacacaaaaaaccaacacacagatctaatgaaaataaagatcttttattgcggcctcaatgctggtccagaatcagtggcacctgggcgctatccactctagggggcagccgttcgccagtgtgcacattaaacataggcagtgtactcagtggccttggcacctccctagaagcagccatctggcgcagttcctcggtgttgccgtgaatagtacaatggtgcaccatctggatatcagatgtggccaggtctctcttcagccgtccctctctccgacagcacatcacataagccagcagcagggtcagcagcagagccaccagcagaggcaccagcagagtcaccagagcgtccaccaggaaatccctgtctggggcttctgttggaggacaaaagaaaggatcgtgctccaggattccgtctccaggggttggcacttcgtcagctggctcaggcacagatttatccaccagagtcacgttgcaccagtccacgcgaaaatggggggccagtgtgtcataacaggacagcagtggtggctgtccctgagcgcacctagcgtgactatcaggagaagccaccatcttcaggcaggtggagaatggggaagcgcttcccactttaatgtacaccccttccttccttccctcgattggcagtggcacccttcctcccctatccagagcgctagtcacattcagcagctgcagttctcctggctcccacagtcctcccagagcggacagaaatctgctggcgggtgttgatggcagcacttcctcagcgtcgtgtgaccgcaccaggaactcggcctgataaggcagcaggggtccttctggatccccaatctccagcaccaggcgctgcctggtagtatcaaaactgtcgcggttgtaagctgtcacttcgatcacctgcagtcccctgtcctctggggtagcgcttccatacaggaatccaggatggtggggtgatctctgggtgtatctcagccaccgtggcagatcaggatggccctgcagatgggcgtggtaagtgatatgcacagcaggtggcacagccacgtgttctggcagactcagaaatgtctcatggtccagggtgtgcacgaacacccggcccaccagtgggtgcagtgtggtctgctgagcctcggtatctcccagtccagccagcagcaccaccagcagaggagtccagaacagtgtctcggccatggtggtaccacgcgctgtaattgaactgggagtggacacctgtggagagaaaggcaaagtggatgtcagtaagaccaataggtgcctatcagaaacgcaagagtcttctctgtctcgacaagcccagtttctattggtctccttaaacctgtcttgtaaccttgatacttacctgcccagtgcctcacgaccaacttctgcaggtgacccgggggcagcccctgtgcccctgggttatatagaggagcctacagggtgtgactagccaggaggggctgtccccagggaggaccagggacagggttatttttagagcgagcttctcctccatggtgtacagagcctaagacccaggcaccggggtggggtaaccgctcaggctcaggcagcaggtgttggggggggggggcagcaggtgttggggttaattataaccaggcatctcgggtgtccccaggccttgcctccttacatgggcagcctagacccgtagtggtccaccagggacagggttatttttagagcgagcttctcctccatggtgtacagagcctaagacccaggcaccggggtggggtaaccgctcaggctcaggcagcaggtgttgggggggggggggcagcaggtgttggggttaattataaccaggcatctcgggtgtccccaggccttgcctccttacatgggcagcatagacccgtagtggatccaccagggacagggttatttttagagcgagcttctcctccatggtgtacagagcctaagacccaggcaccggggtggggtaaccgctcaggctcaggcagcaggtgttgggggggggggggcagcaggtgttggggttaattataaccaggcatctcgggtgtccccaggccttgcctccttacatgggcagcctagacccgtagtggggcatgcaagtttgcggccgccaattggttaaccccactccctctctgcgcgctcgctcgctcactgaggccgcccgggcaaagcccgggcgtcgggcgacctttggtcgcccggcctcagtgagcgagcgagcgcgcagagagggagtggggttaaccaattggcggccgcaaacttgcatgccccactacgggtctaggctgcccatgtaaggaggcaaggcctggggacacccgagatgcctggttataattaaccccaacacctgctgcccccccccccccaacacctgctgcctgagcctgagcggttaccccaccccggtgcctgggtcttaggctctgtacaccatggaggagaagctcgctctaaaaataaccctgtccctggtggatccactacgggtctatgctgcccatgtaaggaggcaaggcctggggacacccgagatgcctggttataattaaccccaacacctgctgcccccccccccccaacacctgctgcctgagcctgagcggttaccccaccccggtgcctgggtcttaggctctgtacaccatggaggagaagctcgctctaaaaataaccctgtccctggtggaccactacgggtctaggctgcccatgtaaggaggcaaggcctggggacacccgagatgcctggttataattaaccccaacacctgctgccccccccccccaacacctgctgcctgagcctgagcggttaccccaccccggtgcctgggtcttaggctctgtacaccatggaggagaagctcgctctaaaaataaccctgtccctggtcctccctggggacagcccctcctggctagtcacaccctgtaggctcctctatataacccaggggcacaggggctgcccccgggtcacctgcagaagttggtcgtgaggcactgggcaggtaagtatcaaggttacaagacaggtttaaggagaccaatagaaactgggcttgtcgagacagagaagactcttgcgtttctgataggcacctattggtcttactgacatccactttgcctttctctccacaggtgtccactcccagttcaattacagcgcgtggtaccaccatggccgagacactgttctggactcctctgctggtggtgctgctggctggactgggagataccgaggctcagcagaccacactgcacccactggtgggccgggtgttcgtgcacaccctggaccatgagacatttctgagtctgccagaacacgtggctgtgccacctgctgtgcatatcacttaccacgcccatctgcagggccatcctgatctgccacggtggctgagatacacccagagatcaccccaccatcctggattcctgtatggaagcgctaccccagaggacaggggactgcaggtgatcgaagtgacagcttacaaccgcgacagttttgatactaccaggcagcgcctggtgctggagattggggatccagaaggacccctgctgccttatcaggccgagttcctggtgcggtcacacgacgctgaggaagtgctgccatcaacacccgccagcagatttctgtccgctctgggaggactgtgggagccaggagaactgcagctgctgaatgtgactagcgctctggataggggaggaagggtgccactgccaatcgagggaaggaaggaaggggtgtacattaaagtgggaagcgcttccccattctccacctgcctgaagatggtggcttctcctgatagtcacgctaggtgcgctcagggacagccaccactgctgtcctgttatgacacactggccccccattttcgcgtggactggtgcaacgtgactctggtggataaatctgtgcctgagccagctgacgaagtgccaacccctggagacggaatcctggagcacgatcctttcttttgtcctccaacagaagccccagacagggatttcctggtggacgctctggtgactctgctggtgcctctgctggtggctctgctgctgaccctgctgctggcttatgtgatgtgctgtcggagagagggacggctgaagagagacctggccacatctgatatccagatggtgcaccattgtactattcacggcaacaccgaggaactgcgccagatggctgcttctagggaggtgccaaggccactgagtacactgcctatgtttaatgtgcacactggcgaacggctgccccctagagtggatagcgcccaggtgccactgattctggaccagcattgaggccgcaataaaagatctttattttcattagatctgtgtgttggttttttgtgtgtcctgcaggggcgcgcctctagagcatggctacgtagataagtagcatggcgggttaatcattaactacaaggaacccctagtgatggagttggccactccctctctgcgcgctcgctcgctcactgaggccgggcgaccaaaggtcgcccgacgcccgggctttgcccgggcggcctcagtgagcgagcgagcgcgcag

SEQ ID NO: 2 - DNA, 1164 bp, synthetic construct
  misc_feature 1..1164: note = hSGCA polynucleotide
  source 1..1164: mol_type = other DNA
atggccgagacactgttctggactcctctgctggtggtgctgctggctggactgggagataccgaggctcagcagaccacactgcacccactggtgggccgggtgttcgtgcacaccctggaccatgagacatttctgagtctgccagaacacgtggctgtgccacctgctgtgcatatcacttaccacgcccatctgcagggccatcctgatctgccacggtggctgagatacacccagagatcaccccaccatcctggattcctgtatggaagcgctaccccagaggacaggggactgcaggtgatcgaagtgacagcttacaaccgcgacagttttgatactaccaggcagcgcctggtgctggagattggggatccagaaggacccctgctgccttatcaggccgagttcctggtgcggtcacacgacgctgaggaagtgctgccatcaacacccgccagcagatttctgtccgctctgggaggactgtgggagccaggagaactgcagctgctgaatgtgactagcgctctggataggggaggaagggtgccactgccaatcgagggaaggaaggaaggggtgtacattaaagtgggaagcgcttccccattctccacctgcctgaagatggtggcttctcctgatagtcacgctaggtgcgctcagggacagccaccactgctgtcctgttatgacacactggccccccattttcgcgtggactggtgcaacgtgactctggtggataaatctgtgcctgagccagctgacgaagtgccaacccctggagacggaatcctggagcacgatcctttcttttgtcctccaacagaagccccagacagggatttcctggtggacgctctggtgactctgctggtgcctctgctggtggctctgctgctgaccctgctgctggcttatgtgatgtgctgtcggagagagggacggctgaagagagacctggccacatctgatatccagatggtgcaccattgtactattcacggcaacaccgaggaactgcgccagatggctgcttctagggaggtgccaaggccactgagtacactgcctatgtttaatgtgcacactggcgaacggctgccccctagagtggatagcgcccaggtgccactgattctggaccagcattga

SEQ ID NO: 3 - protein, 387 aa, synthetic construct
  REGION 1..387: note = hSGCA polypeptide
MAETLFWTPLLVVLLAGLGDTEAQQTTLHPLVGRVFVHTLDHETFLSLPEHVAVPPAVHITYHAHLQGHPDLPRWLRYTQRSPHHPGFLYGSATPEDRGLQVIEVTAYNRDSFDTTRQRLVLEIGDPEGPLLPYQAEFLVRSHDAEEVLPSTPASRFLSALGGLWEPGELQLLNVTSALDRGGRVPLPIEGRKEGVYIKVGSASPFSTCLKMVASPDSHARCAQGQPPLLSCYDTLAPHFRVDWCNVTLVDKSVPEPADEVPTPGDGILEHDPFFCPPTEAPDRDFLVDALVTLLVPLLVALLLTLLLAYVMCCRREGRLKRDLATSDIQMVHHCTIHGNTEELRQMAASREVPRPLSTLPMFNVHTGERLPPRVDSAQVPLILDQH

SEQ ID NO: 4 - DNA, 130 bp, synthetic construct
  misc_feature 1..130: note = complement of 3' ITR
  source 1..130: mol_type = other DNA
ctgcgcgctcgctcgctcactgaggccgcccgggcaaagcccgggcgtcgggcgacctttggtcgcccggcctcagtgagcgagcgagcgcgcagagagggagtggccaactccatcactaggggttcct

SEQ ID NO: 5 - DNA, 53 bp, synthetic construct
  misc_feature 1..53: note = complement of polyA
  source 1..53: mol_type = other DNA
cacaaaaaaccaacacacagatctaatgaaaataaagatcttttattgcggcc

SEQ ID NO: 6 - DNA, 1164 bp, synthetic construct
  misc_feature 1..1164: note = complement of SGCA DNA (SGCA Codon Optimized)
  source 1..1164: mol_type = other DNA
tcaatgctggtccagaatcagtggcacctgggcgctatccactctagggggcagccgttcgccagtgtgcacattaaacataggcagtgtactcagtggccttggcacctccctagaagcagccatctggcgcagttcctcggtgttgccgtgaatagtacaatggtgcaccatctggatatcagatgtggccaggtctctcttcagccgtccctctctccgacagcacatcacataagccagcagcagggtcagcagcagagccaccagcagaggcaccagcagagtcaccagagcgtccaccaggaaatccctgtctggggcttctgttggaggacaaaagaaaggatcgtgctccaggattccgtctccaggggttggcacttcgtcagctggctcaggcacagatttatccaccagagtcacgttgcaccagtccacgcgaaaatggggggccagtgtgtcataacaggacagcagtggtggctgtccctgagcgcacctagcgtgactatcaggagaagccaccatcttcaggcaggtggagaatggggaagcgcttcccactttaatgtacaccccttccttccttccctcgattggcagtggcacccttcctcccctatccagagcgctagtcacattcagcagctgcagttctcctggctcccacagtcctcccagagcggacagaaatctgctggcgggtgttgatggcagcacttcctcagcgtcgtgtgaccgcaccaggaactcggcctgataaggcagcaggggtccttctggatccccaatctccagcaccaggcgctgcctggtagtatcaaaactgtcgcggttgtaagctgtcacttcgatcacctgcagtcccctgtcctctggggtagcgcttccatacaggaatccaggatggtggggtgatctctgggtgtatctcagccaccgtggcagatcaggatggccctgcagatgggcgtggtaagtgatatgcacagcaggtggcacagccacgtgttctggcagactcagaaatgtctcatggtccagggtgtgcacgaacacccggcccaccagtgggtgcagtgtggtctgctgagcctcggtatctcccagtccagccagcagcaccaccagcagaggagtccagaacagtgtctcggccat

SEQ ID NO: 7 - DNA, 714 bp, synthetic construct
  misc_feature 1..714: note = complement of tMCK promoter
  source 1..714: mol_type = other DNA
gtgacccgggggcagcccctgtgcccctgggttatatagaggagcctacagggtgtgactagccaggaggggctgtccccagggaggaccagggacagggttatttttagagcgagcttctcctccatggtgtacagagcctaagacccaggcaccggggtggggtaaccgctcaggctcaggcagcaggtgttggggggggggggcagcaggtgttggggttaattataaccaggcatctcgggtgtccccaggccttgcctccttacatgggcagcctagacccgtagtggtccaccagggacagggttatttttagagcgagcttctcctccatggtgtacagagcctaagacccaggcaccggggtggggtaaccgctcaggctcaggcagcaggtgttgggggggggggggcagcaggtgttggggttaattataaccaggcatctcgggtgtccccaggccttgcctccttacatgggcagcatagacccgtagtggatccaccagggacagggttatttttagagcgagcttctcctccatggtgtacagagcctaagacccaggcaccggggtggggtaaccgctcaggctcaggcagcaggtgttgggggggggggggcagcaggtgttggggttaattataaccaggcatctcgggtgtccccaggccttgcctccttacatgggcagcctagacccgtagtgg

SEQ ID NO: 8 - DNA, 125 bp, synthetic construct
  misc_feature 1..125: note = complement of 5' ITR
  source 1..125: mol_type = other DNA
aaccccactccctctctgcgcgctcgctcgctcactgaggccgcccgggcaaagcccgggcgtcgggcgacctttggtcgcccggcctcagtgagcgagcgagcgcgcagagagggagtggggtt

SEQ ID NO: 9 - DNA, 714 bp, synthetic construct
  misc_feature 1..714: note = tMCK promoter sequence
  source 1..714: mol_type = other DNA
ccactacgggtctaggctgcccatgtaaggaggcaaggcctggggacacccgagatgcctggttataattaaccccaacacctgctgcccccccccccccaacacctgctgcctgagcctgagcggttaccccaccccggtgcctgggtcttaggctctgtacaccatggaggagaagctcgctctaaaaataaccctgtccctggtggatccactacgggtctatgctgcccatgtaaggaggcaaggcctggggacacccgagatgcctggttataattaaccccaacacctgctgcccccccccccccaacacctgctgcctgagcctgagcggttaccccaccccggtgcctgggtcttaggctctgtacaccatggaggagaagctcgctctaaaaataaccctgtccctggtggaccactacgggtctaggctgcccatgtaaggaggcaaggcctggggacacccgagatgcctggttataattaaccccaacacctgctgccccccccccccaacacctgctgcctgagcctgagcggttaccccaccccggtgcctgggtcttaggctctgtacaccatggaggagaagctcgctctaaaaataaccctgtccctggtcctccctggggacagcccctcctggctagtcacaccctgtaggctcctctatataacccaggggcacaggggctgcccccgggtcac

SEQ ID NO: 10 - DNA, 53 bp, synthetic construct
  misc_feature 1..53: note = poly A
  source 1..53: mol_type = other DNA
ggccgcaataaaagatctttattttcattagatctgtgtgttggttttttgtg

SEQ ID NO: 11 - DNA, 130 bp, synthetic construct
  misc_feature 1..130: note = 3' ITR
  source 1..130: mol_type = other DNA
aggaacccctagtgatggagttggccactccctctctgcgcgctcgctcgctcactgaggccgggcgaccaaaggtcgcccgacgcccgggctttgcccgggcggcctcagtgagcgagcgagcgcgcag